European Patent Application EP 4 202 062 A1, published June 28, 2023. Title: USE OF MCM8-cGAS-STING-IFN-I SIGNAL PATHWAY AS DISEASE TARGET. Applicant: GUANGZHOU WOMEN AND CHILDREN'S MEDICAL CENTER. The sequence listing filed with the application follows.

SEQUENCE LISTING (8 sequences)

SEQ ID NO: 1 - RNA, 2523 nt, Homo sapiens
augaauggagaguauagaggcagaggauuuggacgaggaagauuucaaagcuggaaaaggggaagagguggugggaacuucucaggaaaauggagagaaagagaacacagaccugaucugaguaaaaccacaggaaaacguacuucugaacaaaccccacaguuuuugcuuucaacaaagaccccacagucaaugcagucaacauuggaucgauucauaccauauaaaggcuggaagcuuuauuucucugaaguuuacagcgauagcucuccuuugauugagaagauucaagcauuugaaaaauuuuucacaaggcauauugauuuguaugacaaggaugaaauagaaagaaagggaaguauuuugguagauuuuaaagaacugacagaagguggugaaguaacuaacuugauaccagauauagcaacugaacuaagagaugcaccugagaaaaccuuggcuugcauggguuuggcaauacaucagguguuaacuaaggaccuugaaaggcaugcagcugaguuacaagcccaggaaggauugucuaaugauggagaaacaaugguaaaugugccacauauucaugcaaggguguacaacuaugagccuuugacacagcucaagaaugucagagcaaauuacuauggaaaauacauugcucuaagagggacagugguucgugucaguaauauaaagccucuuugcaccaagauggcuuuucuuugugcugcauguggagaaauucagagcuuuccucuuccagauggaaaauacagucuucccacaaaguguccugugccugugugucgaggcaggucauuuacugcucuccgcagcucuccucucacaguuacgauggacuggcagucaaucaaaauccaggaauugaugucugaugaucagagagaagcaggucggauuccacgaacaauagaaugugagcuuguucaugaucuuguggauagcugugucccgggagacacagugacuauuacuggaauugucaaagucucaaaugcggaagaagguucucgaaauaagaaugacaaguguauguuccuuuuguauauugaagcaaauucuauuaguaauagcaaaggacagaaaacaaagaguucugaggauggguguaagcauggaauguugauggaguucucacuuaaagaccuuuaugccauccaagagauucaagcugaagaaaaccuguuuaaacucauugucaacucgcuuugcccugucauuuuuggucaugaacuuguuaaagcagguuuggcauuagcacucuuuggaggaagccagaaauacgcagaugacaaaaacagaauuccaauucggggagacccccacauccuuguuguuggagauccaggccuaggaaaaagucaaaugcuacaggcagcgugcaauguugccccacguggcguguauguuugugguaacaccacgaccaccucuggucugacgguaacucuuucaaaagauaguuccucuggagauuuugcuuuggaagcuggugcccugguacuuggugaucaagguauuuguggaaucgaugaauuugauaagauggggaaucaacaucaagccuuguuggaagccauggagcagcaaaguauuagucuugcuaaggcuggugugguuuguagccuuccugcaagaacuuccauuauugcugcugcaaauccaguuggaggacauuacaauaaagccaaaacaguuucugagaauuuaaaaauggggagugcacuacuauccagauuugauuuggucuuuauccuguuagauacuccaaaugagcaucaugaucacuuacucucugaacaugugauugcaauaagagcuggaaagcagagaaccauuagcagugccacaguagcucguaugaauagucaagauucaaauacuuccguacuugaaguaguuucugagaagccauuaucagaaagacuaaaggugguuccuggagaaacaauagaucccauuccccaccagcuauugagaaaguacauuggcuaugcucggcaguauguguacccaaggcuauccacagaagcugcucgaguucuucaagauuuuuaccuugagcuccggaaacagagccagagguuaaauagcucaccaaucacuaccaggcagcuggaaucuuugauucgucugacagaggcacgagcaagguuggaauugagagaggaagcaaccaaagaagacgcugaggauauaguggaaauuaugaaauauagcaugcuaggaacuuacucugaugaauuugggaaccuagauuuugagcgaucccagcaugguucuggaaugagcaacaggucaacagcgaaaagauuuauuucugcucucaacaacguugcugaaagaacuuauaauaauauauuucaauuucaucaacuucggcagauugccaaagaacuaaacauucagguugcugauuuugaaaauuuuauuggaucacuaaaugaccaggguuaccucuugaaaaaaggcccaaaaguuuaccagcuucaaacuauguaa

SEQ ID NO: 2 - protein, 840 aa, Homo sapiens
MNGEYRGRGFGRGRFQSWKRGRGGGNFSGKWREREHRPDLSKTTGKRTSEQTPQFLLSTKTPQSMQSTLDRFIPYKGWKLYFSEVYSDSSPLIEKIQAFEKFFTRHIDLYDKDEIERKGSILVDFKELTEGGEVTNLIPDIATELRDAPEKTLACMGLAIHQVLTKDLERHAAELQAQEGLSNDGETMVNVPHIHARVYNYEPLTQLKNVRANYYGKYIALRGTVVRVSNIKPLCTKMAFLCAACGEIQSFPLPDGKYSLPTKCPVPVCRGRSFTALRSSPLTVTMDWQSIKIQELMSDDQREAGRIPRTIECELVHDLVDSCVPGDTVTITGIVKVSNAEEGSRNKNDKCMFLLYIEANSISNSKGQKTKSSEDGCKHGMLMEFSLKDLYAIQEIQAEENLFKLIVNSLCPVIFGHELVKAGLALALFGGSQKYADDKNRIPIRGDPHILVVGDPGLGKSQMLQAACNVAPRGVYVCGNTTTTSGLTVTLSKDSSSGDFALEAGALVLGDQGICGIDEFDKMGNQHQALLEAMEQQSISLAKAGVVCSLPARTSIIAAANPVGGHYNKAKTVSENLKMGSALLSRFDLVFILLDTPNEHHDHLLSEHVIAIRAGKQRTISSATVARMNSQDSNTSVLEVVSEKPLSERLKVVPGETIDPIPHQLLRKYIGYARQYVYPRLSTEAARVLQDFYLELRKQSQRLNSSPITTRQLESLIRLTEARARLELREEATKEDAEDIVEIMKYSMLGTYSDEFGNLDFERSQHGSGMSNRSTAKRFISALNNVAERTYNNIFQFHQLRQIAKELNIQVADFENFIGSLNDQGYLLKKGPKVYQLQTM

SEQ ID NO: 3 - DNA, 18 bp, Artificial Sequence
  synthesized
aggucauuuacugcucuc

SEQ ID NO: 4 - protein, 6 aa, Artificial Sequence
  synthesized
RSFTAL

SEQ ID NO: 5 - DNA, 291 bp, Artificial Sequence
  synthesized
cgaggcaggucauuuacugcucuccgcagcucuccucucacaguuacgauggacuggcagucaaucaaaauccaggaauugaugucugaugaucagagagaagcaggucggauuccacgaacaauagaaugugagcuuguucaugaucuuguggauagcugugucccgggagacacagugacuauuacuggaauugucaaagucucaaaugcggaagaagguucucgaaauaagaaugacaaguguauguuccuuuuguauauugaagcaaauucuauuaguaauagcaaa

SEQ ID NO: 6 - DNA, 558 bp, Artificial Sequence
  synthesized
uaugagccuuugacacagcucaagaaugucagagcaaauuacuauggaaaauacauugcucuaagagggacagugguucgugucaguaauauaaagccucuuugcaccaagauggcuuuucuuugugcugcauguggagaaauucagagcuuuccucuuccagauggaaaauacagucuucccacaaaguguccugugccugugugucgaggcaggucauuuacugcucuccgcagcucuccucucacaguuacgauggacuggcagucaaucaaaauccaggaauugaugucugaugaucagagagaagcaggucggauuccacgaacaauagaaugugagcuuguucaugaucuuguggauagcugugucccgggagacacagugacuauuacuggaauugucaaagucucaaaugcggaagaagguucucgaaauaagaaugacaaguguauguuccuuuuguauauugaagcaaauucuauuaguaauagcaaaggacagaaaacaaagaguucugaggauggguguaagcauggaauguugauggaguucuca

SEQ ID NO: 7 - protein, 97 aa, Artificial Sequence
  synthesized
RGRSFTALRSSPLTVTMDWQSIKIQELMSDDQREAGRIPRTIECELVHDLVDSCVPGDTVTITGIVKVSNAEEGSRNKNDKCMFLLYIEANSISNSK

SEQ ID NO: 8 - protein, 186 aa, Artificial Sequence
  synthesized
YEPLTQLKNVRANYYGKYIALRGTVVRVSNIKPLCTKMAFLCAACGEIQSFPLPDGKYSLPTKCPVPVCRGRSFTALRSSPLTVTMDWQSIKIQELMSDDQREAGRIPRTIECELVHDLVDSCVPGDTVTITGIVKVSNAEEGSRNKNDKCMFLLYIEANSISNSKGQKTKSSEDGCKHGMLMEFS